European Patent Application EP 4 524 156 A1, published March 19, 2025. Title: FUSION PROTEIN OF RELAXIN OR ANALOGUE AND MEDICAL USE THEREOF. Applicant: BEIJING TUOJIE BIOPHARMACEUTICAL CO., LTD. Application WO. The sequence listing filed with the application follows.

SEQUENCE LISTING (73 sequences)

SEQ ID NO: 1 - protein, 609 aa, Homo sapiens [sequence omitted]

SEQ ID NO: 2 - protein, 522 aa, synthetic construct
  source 1..522: note = HSA+Avi-his
DAHKSEVAHRFKDLGEENFKALVLIAFAQYLQQCPFEDHVKLVNEVTEFAKTCVADESAENCDKSLHTLFGDKLCTVATLRETYGEMADCCAKQEPERNECFLQHKDDNPNLPRLVRPEVDVMCTAFHDNEETFLKKYLYEIARRHPYFYAPELLFFAKRYKAAFTECCQAADKAACLLPKLDELRDEGKASSAKQRLKCASLQKFGERAFKAWAVARLSQRFPKAEFAEVSKLVTDLTKVHTECCHGDLLECADDRADLAKYICENQDSISSKLKECCEKPLLEKSHCIAEVENDEMPADLPSLAADFVESKDVCKNYAEAKDVFLGMFLYEYARRHPDYSVVLLLRLAKTYETTLEKCCAAADPHECYAKVFDEFKPLVEEPQNLIKQNCELFEQLGEYKFQNALLVRYTKKVPQVSTPTLVEVSRNLGKVGSKCCKHPEAKRMPCAEDYLSVVLNQLCVLHEKTPVSDRVTKCCTESLVNRRPCFSALEVDETGGGGSGLNDIFEAQKIEWHEHHHHHH

SEQ ID NO: 3 - protein, 608 aa, Cynomolgus
MKWVTFISLLFLFSSAYSRGVFRRDTHKSEVAHRFKDLGEEHFKGLVLVAFSQYLQQCPFEEHVKLVNEVTEFAKTCVADESAENCDKSLHTLFGDKLCTVATLRETYGEMADCCAKQEPERNECFLQHKDDNPNLPPLVRPEVDVMCTAFHDNEATFLKKYLYEVARRHPYFYAPELLFFAARYKAAFAECCQAADKAACLLPKLDELRDEGKASSAKQRLKCASLQKFGDRAFKAWAVARLSQKFPKAEFAEVSKLVTDLTKVHTECCHGDLLECADDRADLAKYMCENQDSISSKLKECCDKPLLEKSHCLAEVENDEMPADLPSLAADYVESKDVCKNYAEAKDVFLGMFLYEYARRHPDYSVMLLLRLAKAYEATLEKCCAAADPHECYAKVFDEFQPLVEEPQNLVKQNCELFEQLGEYKFQNALLVRYTKKVPQVSTPTLVEVSRNLGKVGAKCCKLPEAKRMPCAEDYLSVVLNRLCVLHEKTPVSEKVTKCCTESLVNRRPCFSALELDEAYVPKAFNAETFTFHADMCTLSEKEKQVKKQTALVELVKHKPKATKEQLKGVMDNFAAFVEKCCKADDKEACFAEEGPKFVAASQAALA

SEQ ID NO: 4 - protein, 608 aa, Mus musculus
MKWVTFLLLLFVSGSAFSRGVFRREAHKSEIAHRYNDLGEQHFKGLVLIAFSQYLQKCSYDEHAKLVQEVTDFAKTCVADESAANCDKSLHTLFGDKLCAIPNLRENYGELADCCTKQEPERNECFLQHKDDNPSLPPFERPEAEAMCTSFKENPTTFMGHYLHEVARRHPYFYAPELLYYAEQYNEILTQCCAEADKESCLTPKLDGVKEKALVSSVRQRMKCSSMQKFGERAFKAWAVARLSQTFPNADFAEITKLATDLTKVNKECCHGDLLECADDRAELAKYMCENQATISSKLQTCCDKPLLKKAHCLSEVEHDTMPADLPAIAADFVEDQEVCKNYAEAKDVFLGTFLYEYSRRHPDYSVSLLLRLAKKYEATLEKCCAEANPPACYGTVLAEFQPLVEEPKNLVKTNCDLYEKLGEYGFQNAILVRYTQKAPQVSTPTLVEAARNLGRVGTKCCTLPEDQRLPCVEDYLSAILNRVCLLHEKTPVSEHVTKCCSGSLVERRPCFSALTVDETYVPKEFKAETFTFHSDICTLPEKEKQIKKQTALAELVKHKPKATAEQLKTVMDDFAQFLDTCCKAADKDTCFSTEGPNLVTRCKDALA

SEQ ID NO: 5 - protein, 608 aa, Rattus norvegicus
MKWVTFLLLLFISGSAFSRGVFRREAHKSEIAHRFKDLGEQHFKGLVLIAFSQYLQKCPYEEHIKLVQEVTDFAKTCVADENAENCDKSIHTLFGDKLCAIPKLRDNYGELADCCAKQEPERNECFLQHKDDNPNLPPFQRPEAEAMCTSFQENPTSFLGHYLHEVARRHPYFYAPELLYYAEKYNEVLTQCCTESDKAACLTPKLDAVKEKALVAAVRQRMKCSSMQRFGERAFKAWAVARMSQRFPNAEFAEITKLATDVTKINKECCHGDLLECADDRAELAKYMCENQATISSKLQACCDKPVLQKSQCLAEIEHDNIPADLPSIAADFVEDKEVCKNYAEAKDVFLGTFLYEYSRRHPDYSVSLLLRLAKKYEATLEKCCAEGDPPACYGTVLAEFQPLVEEPKNLVKTNCELYEKLGEYGFQNAVLVRYTQKAPQVSTPTLVEAARNLGRVGTKCCTLPEAQRLPCVEDYLSAILNRLCVLHEKTPVSEKVTKCCSGSLVERRPCFSALTVDETYVPKEFKAETFTFHSDICTLPDKEKQIKKQTALAELVKHKPKATEDQLKTVMGDFAQFVDKCCKAADKDNCFATEGPNLVARSKEALA

SEQ ID NO: 6 - protein, 125 aa, synthetic construct
  source 1..125: note = #7aHSA
HVQLVESGGGSVQAGGSLRVSCVASGNTYLTSCMGWFRQAPGKEREGVASIYTVGGSTFYTNSVKGRFTISRDNAKNTVYLQMNSLQPEDTAMYYCAAGSPARCRLRDPTTFDYWGQGTQVTVSS

SEQ ID NO: 7 - protein, 125 aa, synthetic construct
  source 1..125: note = #9aHSA
DVQLVESGGGSVQAGGSLRLSCAAAEYTYLNSCLGWFRQAPGKEREGVATIYMVGGSTFYADSVKGRFTISRDNAKNTVYLMMNSLKPEDTAMYYCAAGSPARCLRRDPTTFNYWGQGTQVTVSS

SEQ ID NO: 8 - protein, 5 aa, synthetic construct
  DOMAIN 1..5: note = CDR
TSCMG

SEQ ID NO: 9 - protein, 17 aa, synthetic construct
  DOMAIN 1..17: note = CDR
SIYTVGGSTFYTNSVKG

SEQ ID NO: 10 - protein, 16 aa, synthetic construct
  DOMAIN 1..16: note = CDR
GSPARCRLRDPTTFDY

SEQ ID NO: 11 - protein, 5 aa, synthetic construct
  DOMAIN 1..5: note = CDR
NSCLG

SEQ ID NO: 12 - protein, 17 aa, synthetic construct
  DOMAIN 1..17: note = CDR
TIYMVGGSTFYADSVKG

SEQ ID NO: 13 - protein, 16 aa, synthetic construct
  DOMAIN 1..16: note = CDR
GSPARCLRRDPTTFNY

SEQ ID NO: 14 - protein, 232 aa, Homo sapiens
EPKSCDKTHTCPPCPAPELLGGPSVFLFPPKPKDTLMISRTPEVTCVVVDVSHEDPEVKFNWYVDGVEVHNAKTKPREEQYNSTYRVVSVLTVLHQDWLNGKEYKCKVSNKALPAPIEKTISKAKGQPREPQVYTLPPSRDELTKNQVSLTCLVKGFYPSDIAVEWESNGQPENNYKTTPPVLDSDGSFFLYSKLTVDKSRWQQGNVFSCSVMHEALHNHYTQKSLSLSPGK

SEQ ID NO: 15 - protein, 361 aa, synthetic construct
  source 1..361: note = #7aHSA-IgG1Fc
HVQLVESGGGSVQAGGSLRVSCVASGNTYLTSCMGWFRQAPGKEREGVASIYTVGGSTFYTNSVKGRFTISRDNAKNTVYLQMNSLQPEDTAMYYCAAGSPARCRLRDPTTFDYWGQGTQVTVSSASGSEPKSCDKTHTCPPCPAPELLGGPSVFLFPPKPKDTLMISRTPEVTCVVVDVSHEDPEVKFNWYVDGVEVHNAKTKPREEQYNSTYRVVSVLTVLHQDWLNGKEYKCKVSNKALPAPIEKTISKAKGQPREPQVYTLPPSRDELTKNQVSLTCLVKGFYPSDIAVEWESNGQPENNYKTTPPVLDSDGSFFLYSKLTVDKSRWQQGNVFSCSVMHEALHNHYTQKSLSLSPGK

SEQ ID NO: 16 - protein, 361 aa, synthetic construct
  source 1..361: note = #9aHSA-IgG1Fc
DVQLVESGGGSVQAGGSLRLSCAAAEYTYLNSCLGWFRQAPGKEREGVATIYMVGGSTFYADSVKGRFTISRDNAKNTVYLMMNSLKPEDTAMYYCAAGSPARCLRRDPTTFNYWGQGTQVTVSSASGSEPKSCDKTHTCPPCPAPELLGGPSVFLFPPKPKDTLMISRTPEVTCVVVDVSHEDPEVKFNWYVDGVEVHNAKTKPREEQYNSTYRVVSVLTVLHQDWLNGKEYKCKVSNKALPAPIEKTISKAKGQPREPQVYTLPPSRDELTKNQVSLTCLVKGFYPSDIAVEWESNGQPENNYKTTPPVLDSDGSFFLYSKLTVDKSRWQQGNVFSCSVMHEALHNHYTQKSLSLSPGK

SEQ ID NO: 17 - protein, 351 aa, synthetic construct
  source 1..351: note = ALB8-IgG1-Fc
EVQLVESGGGLVQPGNSLRLSCAASGFTFSSFGMSWVRQAPGKGLEWVSSISGSGSDTLYADSVKGRFTISRDNAKTTLYLQMNSLRPEDTAVYYCTIGGSLSRSSQGTLVTVSSASGSEPKSCDKTHTCPPCPAPELLGGPSVFLFPPKPKDTLMISRTPEVTCVVVDVSHEDPEVKFNWYVDGVEVHNAKTKPREEQYNSTYRVVSVLTVLHQDWLNGKEYKCKVSNKALPAPIEKTISKAKGQPREPQVYTLPPSRDELTKNQVSLTCLVKGFYPSDIAVEWESNGQPENNYKTTPPVLDSDGSFFLYSKLTVDKSRWQQGNVFSCSVMHEALHNHYTQKSLSLSPGK

SEQ ID NO: 18 - protein, 125 aa, synthetic construct
  source 1..125: note = #7_Hu_1
EVQLLESGGGLVQPGGSLRLSCAASGNTYLTSCMGWFRQAPGKEREGVSSIYTVGGSTFYTNSVKGRFTISRDNSKNTLYLQMNSLRAEDTAVYYCAAGSPARCRLRDPTTFDYWGQGTLVTVSS

SEQ ID NO: 19 - protein, 125 aa, synthetic construct
  source 1..125: note = #7_Hu_2
EVQLLESGGGLVQPGGSLRVSCAASGNTYLTSCMGWFRQAPGKEREGVSSIYTVGGSTFYTNSVKGRFTISRDNSKNTLYLQMNSLRAEDTAVYYCAAGSPARCRLRDPTTFDYWGQGTLVTVSS

SEQ ID NO: 20 - protein, 125 aa, synthetic construct
  source 1..125: note = #7_Hu_3
EVQLLESGGGLVQPGGSLRLSCVASGNTYLTSCMGWFRQAPGKEREGVSSIYTVGGSTFYTNSVKGRFTISRDNSKNTLYLQMNSLRAEDTAVYYCAAGSPARCRLRDPTTFDYWGQGTLVTVSS

SEQ ID NO: 21 - protein, 125 aa, synthetic construct
  source 1..125: note = #7_Hu_4
EVQLLESGGGLVQPGGSLRLSCAASGNTYLTSCMGWFRQAPGKEREGVSSIYTVGGSTFYTNSVKGRFTISRDNAKNTLYLQMNSLRAEDTAVYYCAAGSPARCRLRDPTTFDYWGQGTLVTVSS

SEQ ID NO: 22 - protein, 125 aa, synthetic construct
  source 1..125: note = #7_Hu_5
EVQLLESGGGLVQPGGSLRLSCAASGNTYLTSCMGWFRQAPGKEREGVSSIYTVGGSTFYTNSVKGRFTISRDNSKNTVYLQMNSLRAEDTAVYYCAAGSPARCRLRDPTTFDYWGQGTLVTVSS

SEQ ID NO: 23 - protein, 125 aa, synthetic construct
  source 1..125: note = #7_Hu_6
EVQLLESGGGLVQPGGSLRLSCAASGNTYLTSCMGWFRQAPGKEREGVASIYTVGGSTFYTNSVKGRFTISRDNSKNTLYLQMNSLRAEDTAVYYCAAGSPARCRLRDPTTFDYWGQGTLVTVSS

SEQ ID NO: 24 - protein, 125 aa, synthetic construct
  source 1..125: note = #7_Hu_7
EVQLLESGGGLVQPGGSLRLSCAASGNTYLTSCMGWFRQAPGKEREGVSSIYTVGGSTFYTNSVKGRFTISRDNSKNTLYLQMNSLQPEDTAVYYCAAGSPARCRLRDPTTFDYWGQGTLVTVSS

SEQ ID NO: 25 - protein, 125 aa, synthetic construct
  source 1..125: note = #7_Hu_8
EVQLLESGGGLVQPGGSLRLSCAASGNTYLTSCMGWFRQAPGKEREGVSSIYTVGGSTFYTNSVKGRFTISRDNSKNTLYLQMNSLRPEDTAVYYCAAGSPARCRLRDPTTFDYWGQGTLVTVSS

SEQ ID NO: 26 - protein, 125 aa, synthetic construct
  source 1..125: note = #7_Hu_9
EVQLLESGGGLVQPGGSLRLSCAASGFTFLTSCMGWFRQAPGKEREGVSSIYTVGGSTFYTNSVKGRFTISRDNSKNTLYLQMNSLRPEDTAVYYCAAGSPARCRLRDPTTFDYWGQGTLVTVSS

SEQ ID NO: 27 - protein, 125 aa, synthetic construct
  source 1..125: note = #7_Hu_10
EVQLLESGGGLVQPGGSLRLSCAASGFTFLTSCMGWFRQAPGKEREGVSSIYTVGGSTFYTNSVKGRFTISRDNSKNTLYLQMNSLRAEDTAVYYCAAGSPARCRLRDPTTFDYWGQGTLVTVSS

SEQ ID NO: 28 - protein, 361 aa, synthetic construct
  source 1..361: note = #7_hu_1-hIgG1Fc
EVQLLESGGGLVQPGGSLRLSCAASGNTYLTSCMGWFRQAPGKEREGVSSIYTVGGSTFYTNSVKGRFTISRDNSKNTLYLQMNSLRAEDTAVYYCAAGSPARCRLRDPTTFDYWGQGTLVTVSSASGSEPKSCDKTHTCPPCPAPELLGGPSVFLFPPKPKDTLMISRTPEVTCVVVDVSHEDPEVKFNWYVDGVEVHNAKTKPREEQYNSTYRVVSVLTVLHQDWLNGKEYKCKVSNKALPAPIEKTISKAKGQPREPQVYTLPPSRDELTKNQVSLTCLVKGFYPSDIAVEWESNGQPENNYKTTPPVLDSDGSFFLYSKLTVDKSRWQQGNVFSCSVMHEALHNHYTQKSLSLSPGK

SEQ ID NO: 29 - protein, 140 aa, synthetic construct
  source 1..140: note = #7_Hu_10-6His
EVQLLESGGGLVQPGGSLRLSCAASGFTFLTSCMGWFRQAPGKEREGVSSIYTVGGSTFYTNSVKGRFTISRDNSKNTLYLQMNSLRAEDTAVYYCAAGSPARCRLRDPTTFDYWGQGTLVTVSSGGGGSGGGSHHHHHH

SEQ ID NO: 30 - protein, 130 aa, synthetic construct
  source 1..130: note = ALB8-6his
EVQLVESGGGLVQPGNSLRLSCAASGFTFSSFGMSWVRQAPGKGLEWVSSISGSGSDTLYADSVKGRFTISRDNAKTTLYLQMNSLRPEDTAVYYCTIGGSLSRSSQGTLVTVSSGGGGSGGGSHHHHHH

SEQ ID NO: 31 - protein, 24 aa, synthetic construct
  source 1..24: note = Human RLN2 A chain
QLYSALANKCCHVGCTKRSLARFC

SEQ ID NO: 32 - protein, 28 aa, synthetic construct
  source 1..28: note = Human RLN2 B chain (delB1)
SWMEEVIKLCGRELVRAQIAICGMSTWS

SEQ ID NO: 33 - protein, 25 aa, synthetic construct
  source 1..25: note = Linker
GGGGQGGGGQGGGGQGGGGQGGGGQ

SEQ ID NO: 34 - protein, 32 aa, synthetic construct
  source 1..32: note = Linker
PGPAPGPAPGPAPGPAPGPAPGPAPGPAPGPA

SEQ ID NO: 35 - protein, 32 aa, synthetic construct
  source 1..32: note = Linker
PGPQPGPQPGPQPGPQPGPQPGPQPGPQPGPQ

SEQ ID NO: 36 - protein, 212 aa, synthetic construct
  source 1..212: note = 0051
EVQLLESGGGLVQPGGSLRLSCAASGFTFLTSCMGWFRQAPGKEREGVSSIYTVGGSTFYTNSVKGRFTISRDNSKNTLYLQMNSLRAEDTAVYYCAAGSPARCRLRDPTTFDYWGQGTLVTVSSGGGGQGGGGQGGGGQGGGGQGGGGQSWMEEVIKLCGRELVRAQIAICGMSTWSGGGSGGSGGGQLYSALANKCCHVGCTKRSLARFC

SEQ ID NO: 37 - protein, 219 aa, synthetic construct
  source 1..219: note = 0052
EVQLLESGGGLVQPGGSLRLSCAASGFTFLTSCMGWFRQAPGKEREGVSSIYTVGGSTFYTNSVKGRFTISRDNSKNTLYLQMNSLRAEDTAVYYCAAGSPARCRLRDPTTFDYWGQGTLVTVSSPGPAPGPAPGPAPGPAPGPAPGPAPGPAPGPASWMEEVIKLCGRELVRAQIAICGMSTWSGGGSGGSGGGQLYSALANKCCHVGCTKRSLARFC

SEQ ID NO: 38 - protein, 219 aa, synthetic construct
  source 1..219: note = 0053
EVQLLESGGGLVQPGGSLRLSCAASGFTFLTSCMGWFRQAPGKEREGVSSIYTVGGSTFYTNSVKGRFTISRDNSKNTLYLQMNSLRAEDTAVYYCAAGSPARCRLRDPTTFDYWGQGTLVTVSSPGPQPGPQPGPQPGPQPGPQPGPQPGPQPGPQSWMEEVIKLCGRELVRAQIAICGMSTWSGGGSGGSGGGQLYSALANKCCHVGCTKRSLARFC

SEQ ID NO: 39 - protein, 212 aa, synthetic construct
  source 1..212: note = 0062
EVQLLESGGGLVQPGGSLRLSCAASGNTYLTSCMGWFRQAPGKEREGVSSIYTVGGSTFYTNSVKGRFTISRDNSKNTLYLQMNSLRAEDTAVYYCAAGSPARCRLRDPTTFDYWGQGTLVTVSSGGGGQGGGGQGGGGQGGGGQGGGGQSWMEEVIKLCGRELVRAQIAICGMSTWSGGGSGGSGGGQLYSALANKCCHVGCTKRSLARFC

SEQ ID NO: 40 - protein, 213 aa, synthetic construct
  source 1..213: note = 0063
EVQLLESGGGLVQPGGSLRLSCAASGNTYLTSCMGWFRQAPGKEREGVASIYTVGGSTFYTNSVKGRFTISRDNSKNTLYLQMNSLRAEDTAVYYCAAGSPARCRLRDPTTFDYWGQGTLVTVSSGGGGQGGGGQGGGGQGGGGQGGGGQSWMEEVIKLCGRELVRAQIAICGMSTWSGGGSGGSGGGQLYSALANKCCHVGCTKRSLARFCC

SEQ ID NO: 41 - protein, 212 aa, synthetic construct
  source 1..212: note = 0064
EVQLLESGGGLVQPGGSLRLSCAASGNTYLTSCMGWFRQAPGKEREGVSSIYTVGGSTFYTNSVKGRFTISRDNSKNTLYLQMNSLQPEDTAVYYCAAGSPARCRLRDPTTFDYWGQGTLVTVSSGGGGQGGGGQGGGGQGGGGQGGGGQSWMEEVIKLCGRELVRAQIAICGMSTWSGGGSGGSGGGQLYSALANKCCHVGCTKRSLARFC

SEQ ID NO: 42 - protein, 212 aa, synthetic construct
  source 1..212: note = 0065
EVQLLESGGGLVQPGGSLRLSCAASGFTFLTSCMGWFRQAPGKEREGVSSIYTVGGSTFYTNSVKGRFTISRDNSKNTLYLQMNSLRPEDTAVYYCAAGSPARCRLRDPTTFDYWGQGTLVTVSSGGGGQGGGGQGGGGQGGGGQGGGGQSWMEEVIKLCGRELVRAQIAICGMSTWSGGGSGGSGGGQLYSALANKCCHVGCTKRSLARFC

SEQ ID NO: 43 - protein, 212 aa, synthetic construct
  source 1..212: note = 0066
EVQLLESGGGLVQPGGSLRLSCAASGNTYLTSCMGWFRQAPGKEREGVSSIYTVGGSTFYTNSVKGRFTISRDNSKNTLYLQMNSLRPEDTAVYYCAAGSPARCRLRDPTTFDYWGQGTLVTVSSGGGGQGGGGQGGGGQGGGGQGGGGQSWMEEVIKLCGRELVRAQIAICGMSTWSGGGSGGSGGGQLYSALANKCCHVGCTKRSLARFC

SEQ ID NO: 44 - protein, 213 aa, synthetic construct
  source 1..213: note = 0054
EVQLLESGGGLVQPGGSLRLSCAASGRYIDETAVAWFRQAPGKGREFVAGIGGGVDITYYADSVKGRFTISRDNSKNTLYLQMNSLRPEDTAVYYCAARPGRPLITSKVADLYPYWGQGTLVTVSSGGGGQGGGGQGGGGQGGGGQGGGGQSWMEEVIKLCGRELVRAQIAICGMSTWSGGGSGGSGGGQLYSALANKCCHVGCTKRSLARFC

SEQ ID NO: 45 - protein, 24 aa, synthetic construct
  source 1..24: note = A chain of 800814
DLYSALANKCCHVGCTKRSLARFC

SEQ ID NO: 46 - protein, 29 aa, synthetic construct
  source 1..29: note = B chain of 800814
DSWMEEVIKLCGRDLVRAQIAICGMSTWS

SEQ ID NO: 47 - protein, 271 aa, synthetic construct
  source 1..271: note = A chain of 0060
DKTHTCPPCPAPEFEGGPSVFLFPPKPKDTLMISRTPEVTCVVVDVSHEDPEVKFNWYVDGVEVHNAKTKPREEQYNSTYRVVSVLTVLHQDWLNGKEYKCKVSNKALPASIEKTISKAKGQPREPQVYTLPPCREEMTKNQVSLWCLVKGFYPSDIAVEWESNGQPENNYKTTPPVLDSDGSFFLYSKLTVDKSRWQQGNVFSCSVMHEALHNHYTQKSLSLSPGGGGGSGGGGSGGGGSGGGGGSQLYSALANKCCHVGCTKRSLARFC

SEQ ID NO: 48 - protein, 275 aa, synthetic construct
  source 1..275: note = B chain of 0060
DKTHTCPPCPAPEFEGGPSVFLFPPKPKDTLMISRTPEVTCVVVDVSHEDPEVKFNWYVDGVEVHNAKTKPREEQYNSTYRVVSVLTVLHQDWLNGKEYKCKVSNKALPASIEKTISKAKGQPREPQVCTLPPSREEMTKNQVSLSCAVKGFYPSDIAVEWESNGQPENNYKTTPPVLDSDGSFFLVSKLTVDKSRWQQGNVFSCSVMHEALHNHYTQKSLSLSPGGGGGSGGGGSGGGGSGGGGGSSWMEEVIKLCGRELVRAQIAICGMSTWS

SEQ ID NO: 49 - protein, 10 aa, synthetic construct
  source 1..10: note = Linker
GGGSGGSGGG

SEQ ID NO: 50 - protein, 23 aa, synthetic construct
  source 1..23: note = Human RLN1 A chain
PYVALFEKCCLIGCTKRSLAKYC

SEQ ID NO: 51 - protein, 31 aa, synthetic construct
  source 1..31: note = Human RLN1 B chain
VAAKWKDDVIKLCGRELVRAQIAICGMSTWS

SEQ ID NO: 52 - protein, 20 aa, synthetic construct
  source 1..20: note = Human RLN2 A chain (delA1-4)
ALANKCCHVGCTKRSLARFC

SEQ ID NO: 53 - protein, 29 aa, synthetic construct
  source 1..29: note = Human RLN2 B chain
DSWMEEVIKLCGRELVRAQIAICGMSTWS

SEQ ID NO: 54 - protein, 24 aa, synthetic construct
  source 1..24: note = Human RLN3 A chain
DVLAGLSSSCCKWGCSKSEISSLC

SEQ ID NO: 55 - protein, 27 aa, synthetic construct
  source 1..27: note = Human RLN3 B chain
RAAPYGVRLCGREFIRAVIFTCGGSRW

SEQ ID NO: 56 - protein, 24 aa, synthetic construct
  VARIANT 1: note = X is Q or D
XLYSALANKCCHVGCTKRSLARFC

SEQ ID NO: 57 - protein, 29 aa, synthetic construct
  source 1..29: note = Human RLN2 B chain (E mutated to D)
DSWMEEVIKLCGRDLVRAQIAICGMSTWS

SEQ ID NO: 58 - protein, 17 aa, synthetic construct
  VARIANT 1: note = X is S or T
  VARIANT 4: note = X is T or M
  VARIANT 12: note = X is T or A
  VARIANT 13: note = X is N or D
XIYXVGGSTFYXXSVKG

SEQ ID NO: 59 - protein, 16 aa, synthetic construct
  VARIANT 7: note = X is R or L
  VARIANT 8: note = X is L or R
  VARIANT 15: note = X is D or N
GSPARCXXRDPTTFXY

SEQ ID NO: 60 - protein, 8 aa, synthetic construct
  PEPTIDE 1..8: note = linker
KRGGGPRR

SEQ ID NO: 61 - protein, 8 aa, synthetic construct
  PEPTIDE 1..8: note = linker
KRGGGPKR

SEQ ID NO: 62 - protein, 11 aa, synthetic construct
  PEPTIDE 1..11: note = linker
KRKPTGYGSKR

SEQ ID NO: 63 - protein, 6 aa, synthetic construct
  PEPTIDE 1..6: note = linker
KRSLKR

SEQ ID NO: 64 - skipped

SEQ ID NO: 65 - protein, 13 aa, synthetic construct
  PEPTIDE 1..13: note = linker
KRKPTGYGSRKKR

SEQ ID NO: 66 - protein, 12 aa, synthetic construct
  PEPTIDE 1..12: note = linker
KRKPTGYGSRKR

SEQ ID NO: 67 - protein, 5 aa, synthetic construct
  PEPTIDE 1..5: note = linker
GGGGS

SEQ ID NO: 68 - protein, 10 aa, synthetic construct
  PEPTIDE 1..10: note = linker
GGGGSGGGGS

SEQ ID NO: 69 - protein, 15 aa, synthetic construct
  PEPTIDE 1..15: note = linker
GGGGSGGGGSGGGGS

SEQ ID NO: 70 - protein, 20 aa, synthetic construct
  PEPTIDE 1..20: note = linker
GGGGSGGGGSGGGGSGGGGS

SEQ ID NO: 71 - protein, 25 aa, synthetic construct
  PEPTIDE 1..25: note = linker
GGGGSGGGGSGGGGSGGGGSGGGGS

SEQ ID NO: 72 - protein, 9 aa, synthetic construct
  PEPTIDE 1..9: note = linker
GGGGSGGGS

SEQ ID NO: 73 - protein, 5 aa, synthetic construct
  source 1..5: note = linker
GGGGQ